European Patent Application EP 4 632 120 A2, published October 15, 2025. Title: LIBRARY OF ANTIGEN-BINDING MOLECULES INCLUDING MODIFIED ANTIBODY VARIABLE REGION. Applicant: CHUGAI SEIYAKU KABUSHIKI KAISHA. Application EP. The sequence listing filed with the application follows.

SEQUENCE LISTING (136 sequences)

SEQ ID NO: 1 - protein, 330 aa, Homo sapiens [sequence omitted]

SEQ ID NO: 2 - protein, 326 aa, Homo sapiens
ASTKGPSVFPLAPCSRSTSESTAALGCLVKDYFPEPVTVSWNSGALTSGVHTFPAVLQSSGLYSLSSVVTVPSSNFGTQTYTCNVDHKPSNTKVDKTVERKCCVECPPCPAPPVAGPSVFLFPPKPKDTLMISRTPEVTCVVVDVSHEDPEVQFNWYVDGVEVHNAKTKPREEQFNSTFRVVSVLTVVHQDWLNGKEYKCKVSNKGLPAPIEKTISKTKGQPREPQVYTLPPSREEMTKNQVSLTCLVKGFYPSDIAVEWESNGQPENNYKTTPPMLDSDGSFFLYSKLTVDKSRWQQGNVFSCSVMHEALHNHYTQKSLSLSPGK

SEQ ID NO: 3 - protein, 377 aa, Homo sapiens
ASTKGPSVFPLAPCSRSTSGGTAALGCLVKDYFPEPVTVSWNSGALTSGVHTFPAVLQSSGLYSLSSVVTVPSSSLGTQTYTCNVNHKPSNTKVDKRVELKTPLGDTTHTCPRCPEPKSCDTPPPCPRCPEPKSCDTPPPCPRCPEPKSCDTPPPCPRCPAPELLGGPSVFLFPPKPKDTLMISRTPEVTCVVVDVSHEDPEVQFKWYVDGVEVHNAKTKPREEQYNSTFRVVSVLTVLHQDWLNGKEYKCKVSNKALPAPIEKTISKTKGQPREPQVYTLPPSREEMTKNQVSLTCLVKGFYPSDIAVEWESSGQPENNYNTTPPMLDSDGSFFLYSKLTVDKSRWQQGNIFSCSVMHEALHNRFTQKSLSLSPGK

SEQ ID NO: 4 - protein, 327 aa, Homo sapiens
ASTKGPSVFPLAPCSRSTSESTAALGCLVKDYFPEPVTVSWNSGALTSGVHTFPAVLQSSGLYSLSSVVTVPSSSLGTKTYTCNVDHKPSNTKVDKRVESKYGPPCPSCPAPEFLGGPSVFLFPPKPKDTLMISRTPEVTCVVVDVSQEDPEVQFNWYVDGVEVHNAKTKPREEQFNSTYRVVSVLTVLHQDWLNGKEYKCKVSNKGLPSSIEKTISKAKGQPREPQVYTLPPSQEEMTKNQVSLTCLVKGFYPSDIAVEWESNGQPENNYKTTPPVLDSDGSFFLYSRLTVDKSRWQEGNVFSCSVMHEALHNHYTQKSLSLSLGK

SEQ ID NO: 5 - protein, 4 aa, synthetic construct
  REGION 1..4: note = An artificially synthesized peptide sequence
GGGS

SEQ ID NO: 6 - protein, 4 aa, synthetic construct
  REGION 1..4: note = An artificially synthesized peptide sequence
SGGG

SEQ ID NO: 7 - protein, 5 aa, synthetic construct
  REGION 1..5: note = An artificially synthesized peptide sequence
GGGGS

SEQ ID NO: 8 - protein, 5 aa, synthetic construct
  REGION 1..5: note = An artificially synthesized peptide sequence
SGGGG

SEQ ID NO: 9 - protein, 6 aa, synthetic construct
  REGION 1..6: note = An artificially synthesized peptide sequence
GGGGGS

SEQ ID NO: 10 - protein, 6 aa, synthetic construct
  REGION 1..6: note = An artificially synthesized peptide sequence
SGGGGG

SEQ ID NO: 11 - protein, 7 aa, synthetic construct
  REGION 1..7: note = An artificially synthesized peptide sequence
GGGGGGS

SEQ ID NO: 12 - protein, 7 aa, synthetic construct
  REGION 1..7: note = An artificially synthesized peptide sequence
SGGGGGG

SEQ ID NO: 13 - protein, 122 aa, Rattus norvegicus
EVQLVETGGSLVQPGKSLKLTCATSGFTFSNAWMHWVRQSPEKQLEWVAQIKAKSNNYATYYAESVKGRFTISRDDSKSNIYLQMNSLKEEDTAVYYCRYVHYGAYYGVDAWGQGTSVTVSS

SEQ ID NO: 14 - protein, 112 aa, Rattus norvegicus
DVVMTQTPVSMSVSLGGQVSISCRSSQSLVHNNGNTYVSWYIQKPSQSPQLLIYKVSNRFSGISDRFSGSGSGTDFTLKISRVEPDDLGVYYCGQGTQDPYTFGAGTKLELK

SEQ ID NO: 15 - protein, 119 aa, Mus musculus
QVQLKQSGPGLVQPSQSLSITCTVSGFSLTNYGVHWVRQSPGKGLEWLGVIWSGGNTDYNTPFTSRLSINKDNSKSQVFFKMNSLQSNDTAIYYCARALTYYDYEFAYWGQGTLVTVSA

SEQ ID NO: 16 - protein, 107 aa, Mus musculus
DILLTQSPVILSVSPGERVSFSCRASQSIGTNIHWYQQRTNGSPRLLIKYASESISGIPSRFSGSGSGTDFTLSINSVESEDIADYYCQQNNNWPTTFGAGTKLELK

SEQ ID NO: 17 - protein, 447 aa, synthetic construct
  REGION 1..447: note = An artificially synthesized peptide sequence
QVQLKQSGPGLVQPSQSLSITCTVSGFSLTNYGVHWVRQSPGKGLEWLGVIWSGGNTDYNTPFTSRLSINKDNSKSQVFFKMNSLQSNDTAIYYCARALTYYDYEFAYWGQGTLVTVSAASTKGPSVFPLAPSSKSTSGGTAALGCLVKDYFPEPVTVSWNSGALTSGVHTFPAVLQSSGLYSLSSVVTVPSSSLGTQTYICNVNHKPSNTKVDKKVEPKSCDKTHTCPPCPAPELLGGPSVFLFPPKPKDTLMISRTPEVTCVVVDVSHEDPEVKFNWYVDGVEVHNAKTKPREEQYNSTYRVVSVLTVLHQDWLNGKEYKCKVSNKALPAPIEKTISKAKGQPREPQVYTLPPSRDELTKNQVSLTCLVKGFYPSDIAVEWESNGQPENNYKTTPPVLDSDGSFFLYSKLTVDKSRWQQGNVFSCSVMHEALHNHYTQKSLSLSP

SEQ ID NO: 18 - protein, 447 aa, synthetic construct
  REGION 1..447: note = An artificially synthesized peptide sequence
QVQLKQSGPGLVQPSQSLSITCTVSGFSLTNYGVHWVRQSPGKGLEWLGVIWSGGNTDYNTPFTSRLSINKDNSKSQVFFKMNSLQSNDTAIYYCARALTYYDYEFAYWGQGTLVTVSAASTKGPSVFPLAPSSKSTSGGTAALGCLVKDYFPEPVTVSWNSGALTSGVHTFPAVLQSSGLYSLSSVVTVPSSSLGTQTYICNVNHKPSNTKVDKKVEPKSCDKTHTCPPCPAPELLGGPSVFLFPPKPKDTLMISRTPEVTCVVVDVSHEDPEVKFNWYVDGVEVHNAKTKPREEQYNSTYRVVSVLTVLHQDWLNGKEYKCKVSNKALPAPIEKTISKAKGQPREPQVYTLPPSRKELTKNQVSLTCLVKGFYPSDIAVEWESNGQPENNYKTTPPVLDSDGSFFLYSKLTVDKSRWQQGNVFSCSVMHEALHNRYTQKSLSLSP

SEQ ID NO: 19 - protein, 447 aa, synthetic construct
  REGION 1..447: note = An artificially synthesized peptide sequence
QVQLKQSGPGLVQPSQSLSITCTVSGFSLTNYGVHWVRQSPGKGLEWLGVIWSGGNTDYNTPFTSRLSINKDNSKSQVFFKMNSLQSNDTAIYYCARALTYYDYEFAYWGQGTLVTVSAASTKGPSVFPLAPSSKSTSGGTAALGCLVKDYFPEPVTVSWNSGALTSGVHTFPAVLQSSGLYSLSSVVTVPSSSLGTQTYICNVNHKPSNTKVDKKVEPKSCDKTHTCPPCPAPELLGGPSVFLFPPKPKDTLMISRTPEVTCVVVDVSHEDPEVKFNWYVDGVEVHNAKTKPREEQYNSTYRVVSVLTVLHQDWLNGKEYKCKVSNKALPAPIEKTISKAKGQPREPQVYTLPPSRDELTKNQVSLTCLVKGFYPSDIAVEWESNGQPENNYKTTPPVLDSDGSFFLYSKLTVDKSRWQQGNVFSCSVMHEALHNHYTQESLSLSP

SEQ ID NO: 20 - protein, 445 aa, synthetic construct
  REGION 1..445: note = An artificially synthesized peptide sequence
DILLTQSPVILSVSPGERVSFSCRASQSIGTNIHWYQQRTNGSPRLLIKYASESISGIPSRFSGSGSGTDFTLSINSVESEDIADYYCQQNNNWPTTFGAGTKLELKSSASTKGPSVFPLAPSSKSTSGGTAALGCLVKDYFPEPVTVSWNSGALTSGVHTFPAVLQSSGLYSLSSVVTVPSSSLGTQTYICNVNHKPSNTKVDKKVEPKSCDKTHTCPPCPAPEAAGGPSVFLFPPKPKDTLMISRTPEVTCVVVDVSHEDPEVKFNWYVDGVEVHNAKTKPREEQYASTYRVVSVLTVLHQDWLNGKEYKCKVSNKALPAPIEKTISKAKGQPREPQVCTLPPSRDELTKNQVSLWCLVKGFYPSDIAVEWESNGQPENNYKTTPPVLDSDGSFFLYSKLTVDKSRWQQGNVFSCSVMHEALHNRYTQKSLSLSPHHHHHHHH

SEQ ID NO: 21 - protein, 226 aa, synthetic construct
  REGION 1..226: note = An artificially synthesized peptide sequence
QVQLKQSGPGLVQPSQSLSITCTVSGFSLTNYGVHWVRQSPGKGLEWLGVIWSGGNTDYNTPFTSRLSINKDNSKSQVFFKMNSLQSNDTAIYYCARALTYYDYEFAYWGQGTLVTVSARTVAAPSVFIFPPSDEQLKSGTASVVCLLNNFYPREAKVQWKVDNALQSGNSQESVTEQDSKDSTYSLSSTLTLSKADYEKHKVYACEVTHQGLSSPVTKSFNRGEC

SEQ ID NO: 22 - protein, 458 aa, synthetic construct
  REGION 1..458: note = An artificially synthesized peptide sequence
EVQLVETGGSLVQPGKSLKLTCATSGFTFSNAWMHWVRQSPEKQLEWVAQIKAKSNNYATYYAESVKGRFTISRDDSKSNIYLQMNSLKEEDTAVYYCRYVHYGAYYGVDAWGQGTSVTVSSASTKGPSVFPLAPSSKSTSGGTAALGCLVKDYFPEPVTVSWNSGALTSGVHTFPAVLQSSGLYSLSSVVTVPSSSLGTQTYICNVNHKPSNTKVDKKVEPKSCDKTHTCPPCPAPEAAGGPSVFLFPPKPKDTLMISRTPEVTCVVVDVSHEDPEVKFNWYVDGVEVHNAKTKPREEQYASTYRVVSVLTVLHQDWLNGKEYKCKVSNKALPAPIEKTISKAKGQPREPQVYTLPPSRCELTKNQVSLSCAVKGFYPSDIAVEWESNGQPENNYKTTPPVLDSDGSFFLVSKLTVDKSRWQQGNVFSCSVMHEALHNHYTQKSLSLSPDYKDDDDK

SEQ ID NO: 23 - protein, 219 aa, synthetic construct
  REGION 1..219: note = An artificially synthesized peptide sequence
DVVMTQTPVSMSVSLGGQVSISCRSSQSLVHNNGNTYVSWYIQKPSQSPQLLIYKVSNRFSGISDRFSGSGSGTDFTLKISRVEPDDLGVYYCGQGTQDPYTFGAGTKLELKRTVAAPSVFIFPPSDEQLKSGTASVVCLLNNFYPREAKVQWKVDNALQSGNSQESVTEQDSKDSTYSLSSTLTLSKADYEKHKVYACEVTHQGLSSPVTKSFNRGEC

SEQ ID NO: 24 - protein, 462 aa, synthetic construct
  REGION 1..462: note = An artificially synthesized peptide sequence
EVQLVETGGSLVQPGKSLKLTCATSGFTFSNAWMHWVRQSPEKQLEWVAQIKAGCRGDCLNYATYYAESVKGRFTISRDDSKSNIYLQMNSLKEEDTAVYYCRYVHYGAYYGVDAWGQGTSVTVSSASTKGPSVFPLAPSSKSTSGGTAALGCLVKDYFPEPVTVSWNSGALTSGVHTFPAVLQSSGLYSLSSVVTVPSSSLGTQTYICNVNHKPSNTKVDKKVEPKSCDKTHTCPPCPAPEAAGGPSVFLFPPKPKDTLMISRTPEVTCVVVDVSHEDPEVKFNWYVDGVEVHNAKTKPREEQYASTYRVVSVLTVLHQDWLNGKEYKCKVSNKALPAPIEKTISKAKGQPREPQVYTLPPSRCELTKNQVSLSCAVKGFYPSDIAVEWESNGQPENNYKTTPPVLDSDGSFFLVSKLTVDKSRWQQGNVFSCSVMHEALHNHYTQKSLSLSPDYKDDDDK

SEQ ID NO: 25 - protein, 462 aa, synthetic construct
  REGION 1..462: note = An artificially synthesized peptide sequence
EVQLVETGGSLVQPGKSLKLTCATSGFTFSNAWMHWVRQSPEKQLEWVAQIKAKGCRGDCLYATYYAESVKGRFTISRDDSKSNIYLQMNSLKEEDTAVYYCRYVHYGAYYGVDAWGQGTSVTVSSASTKGPSVFPLAPSSKSTSGGTAALGCLVKDYFPEPVTVSWNSGALTSGVHTFPAVLQSSGLYSLSSVVTVPSSSLGTQTYICNVNHKPSNTKVDKKVEPKSCDKTHTCPPCPAPEAAGGPSVFLFPPKPKDTLMISRTPEVTCVVVDVSHEDPEVKFNWYVDGVEVHNAKTKPREEQYASTYRVVSVLTVLHQDWLNGKEYKCKVSNKALPAPIEKTISKAKGQPREPQVYTLPPSRCELTKNQVSLSCAVKGFYPSDIAVEWESNGQPENNYKTTPPVLDSDGSFFLVSKLTVDKSRWQQGNVFSCSVMHEALHNHYTQKSLSLSPDYKDDDDK

SEQ ID NO: 26 - protein, 465 aa, synthetic construct
  REGION 1..465: note = An artificially synthesized peptide sequence
EVQLVETGGSLVQPGKSLKLTCATSGFTFSNAWMHWVRQSPEKQLEWVAQIKAGCRGDCLKSNNYATYYAESVKGRFTISRDDSKSNIYLQMNSLKEEDTAVYYCRYVHYGAYYGVDAWGQGTSVTVSSASTKGPSVFPLAPSSKSTSGGTAALGCLVKDYFPEPVTVSWNSGALTSGVHTFPAVLQSSGLYSLSSVVTVPSSSLGTQTYICNVNHKPSNTKVDKKVEPKSCDKTHTCPPCPAPEAAGGPSVFLFPPKPKDTLMISRTPEVTCVVVDVSHEDPEVKFNWYVDGVEVHNAKTKPREEQYASTYRVVSVLTVLHQDWLNGKEYKCKVSNKALPAPIEKTISKAKGQPREPQVYTLPPSRCELTKNQVSLSCAVKGFYPSDIAVEWESNGQPENNYKTTPPVLDSDGSFFLVSKLTVDKSRWQQGNVFSCSVMHEALHNHYTQKSLSLSPDYKDDDDK

SEQ ID NO: 27 - protein, 465 aa, synthetic construct
  REGION 1..465: note = An artificially synthesized peptide sequence
EVQLVETGGSLVQPGKSLKLTCATSGFTFSNAWMHWVRQSPEKQLEWVAQIKAKGCRGDCLSNNYATYYAESVKGRFTISRDDSKSNIYLQMNSLKEEDTAVYYCRYVHYGAYYGVDAWGQGTSVTVSSASTKGPSVFPLAPSSKSTSGGTAALGCLVKDYFPEPVTVSWNSGALTSGVHTFPAVLQSSGLYSLSSVVTVPSSSLGTQTYICNVNHKPSNTKVDKKVEPKSCDKTHTCPPCPAPEAAGGPSVFLFPPKPKDTLMISRTPEVTCVVVDVSHEDPEVKFNWYVDGVEVHNAKTKPREEQYASTYRVVSVLTVLHQDWLNGKEYKCKVSNKALPAPIEKTISKAKGQPREPQVYTLPPSRCELTKNQVSLSCAVKGFYPSDIAVEWESNGQPENNYKTTPPVLDSDGSFFLVSKLTVDKSRWQQGNVFSCSVMHEALHNHYTQKSLSLSPDYKDDDDK

SEQ ID NO: 28 - protein, 465 aa, synthetic construct
  REGION 1..465: note = An artificially synthesized peptide sequence
EVQLVETGGSLVQPGKSLKLTCATSGFTFSNAWMHWVRQSPEKQLEWVAQIKAKSNNYATYYAESVKGRFTISRDGCRGDCLDSKSNIYLQMNSLKEEDTAVYYCRYVHYGAYYGVDAWGQGTSVTVSSASTKGPSVFPLAPSSKSTSGGTAALGCLVKDYFPEPVTVSWNSGALTSGVHTFPAVLQSSGLYSLSSVVTVPSSSLGTQTYICNVNHKPSNTKVDKKVEPKSCDKTHTCPPCPAPEAAGGPSVFLFPPKPKDTLMISRTPEVTCVVVDVSHEDPEVKFNWYVDGVEVHNAKTKPREEQYASTYRVVSVLTVLHQDWLNGKEYKCKVSNKALPAPIEKTISKAKGQPREPQVYTLPPSRCELTKNQVSLSCAVKGFYPSDIAVEWESNGQPENNYKTTPPVLDSDGSFFLVSKLTVDKSRWQQGNVFSCSVMHEALHNHYTQKSLSLSPDYKDDDDK

SEQ ID NO: 29 - protein, 463 aa, synthetic construct
  REGION 1..463: note = An artificially synthesized peptide sequence
EVQLVETGGSLVQPGKSLKLTCATSGFTFSNAWMHWVRQSPEKQLEWVAQIKAGCRGDCLNNYATYYAESVKGRFTISRDDSKSNIYLQMNSLKEEDTAVYYCRYVHYGAYYGVDAWGQGTSVTVSSASTKGPSVFPLAPSSKSTSGGTAALGCLVKDYFPEPVTVSWNSGALTSGVHTFPAVLQSSGLYSLSSVVTVPSSSLGTQTYICNVNHKPSNTKVDKKVEPKSCDKTHTCPPCPAPEAAGGPSVFLFPPKPKDTLMISRTPEVTCVVVDVSHEDPEVKFNWYVDGVEVHNAKTKPREEQYASTYRVVSVLTVLHQDWLNGKEYKCKVSNKALPAPIEKTISKAKGQPREPQVYTLPPSRCELTKNQVSLSCAVKGFYPSDIAVEWESNGQPENNYKTTPPVLDSDGSFFLVSKLTVDKSRWQQGNVFSCSVMHEALHNHYTQKSLSLSPDYKDDDDK

SEQ ID NO: 30 - protein, 465 aa, synthetic construct
  REGION 1..465: note = An artificially synthesized peptide sequence
EVQLVETGGSLVQPGKSLKLTCATSGFTFSNAWMHWVRQSPEKQLEWVAQIKAKSNNYATYYAESVKGRFTISRDDSKSNIYLQMNSLKEEDTAVYYCRYVHYGGCRGDCLAYYGVDAWGQGTSVTVSSASTKGPSVFPLAPSSKSTSGGTAALGCLVKDYFPEPVTVSWNSGALTSGVHTFPAVLQSSGLYSLSSVVTVPSSSLGTQTYICNVNHKPSNTKVDKKVEPKSCDKTHTCPPCPAPEAAGGPSVFLFPPKPKDTLMISRTPEVTCVVVDVSHEDPEVKFNWYVDGVEVHNAKTKPREEQYASTYRVVSVLTVLHQDWLNGKEYKCKVSNKALPAPIEKTISKAKGQPREPQVYTLPPSRCELTKNQVSLSCAVKGFYPSDIAVEWESNGQPENNYKTTPPVLDSDGSFFLVSKLTVDKSRWQQGNVFSCSVMHEALHNHYTQKSLSLSPDYKDDDDK

SEQ ID NO: 31 - protein, 465 aa, synthetic construct
  REGION 1..465: note = An artificially synthesized peptide sequence
EVQLVETGGSLVQPGKSLKLTCATSGFTFSNAWMHWVRQSPEKQLEWVAQIKAKSNNYATYYAESVKGRFTISRDDSKSNIYLQMNSLKEEDTAVYYCRYVHYGAGCRGDCLYYGVDAWGQGTSVTVSSASTKGPSVFPLAPSSKSTSGGTAALGCLVKDYFPEPVTVSWNSGALTSGVHTFPAVLQSSGLYSLSSVVTVPSSSLGTQTYICNVNHKPSNTKVDKKVEPKSCDKTHTCPPCPAPEAAGGPSVFLFPPKPKDTLMISRTPEVTCVVVDVSHEDPEVKFNWYVDGVEVHNAKTKPREEQYASTYRVVSVLTVLHQDWLNGKEYKCKVSNKALPAPIEKTISKAKGQPREPQVYTLPPSRCELTKNQVSLSCAVKGFYPSDIAVEWESNGQPENNYKTTPPVLDSDGSFFLVSKLTVDKSRWQQGNVFSCSVMHEALHNHYTQKSLSLSPDYKDDDDK

SEQ ID NO: 32 - protein, 465 aa, synthetic construct
  REGION 1..465: note = An artificially synthesized peptide sequence
EVQLVETGGSLVQPGKSLKLTCATSGFTFSNAWMHWVRQSPEKQLEWVAQIKAKSNNYATYYAESVKGRFTISRDDSKSNIYLQMNSLKEEDTAVYYCRYVHYGAYGCRGDCLYGVDAWGQGTSVTVSSASTKGPSVFPLAPSSKSTSGGTAALGCLVKDYFPEPVTVSWNSGALTSGVHTFPAVLQSSGLYSLSSVVTVPSSSLGTQTYICNVNHKPSNTKVDKKVEPKSCDKTHTCPPCPAPEAAGGPSVFLFPPKPKDTLMISRTPEVTCVVVDVSHEDPEVKFNWYVDGVEVHNAKTKPREEQYASTYRVVSVLTVLHQDWLNGKEYKCKVSNKALPAPIEKTISKAKGQPREPQVYTLPPSRCELTKNQVSLSCAVKGFYPSDIAVEWESNGQPENNYKTTPPVLDSDGSFFLVSKLTVDKSRWQQGNVFSCSVMHEALHNHYTQKSLSLSPDYKDDDDK

SEQ ID NO: 33 - protein, 444 aa, synthetic construct
  REGION 1..444: note = An artificially synthesized peptide sequence
QDQLVQSGAEVKKPGASVKVSCKASGFNIKDTYIQWVRQAPGQGLEWMGRIDPLRKQTKYREKFEGRVTITADTSTNTAYMELSSLRSEDTAVYYCVRSGREFDYWGQGTLVTVSSASTKGPSVFPLAPSSKSTSGGTAALGCLVKDYFPEPVTVSWNSGALTSGVHTFPAVLQSSGLYSLSSVVTVPSSSLGTQTYICNVNHKPSNTKVDKKVEPKSCDKTHTCPPCPAPEYQWGPMVFLFPPKPKDTLMISRTPEVTCVVVDVSDEEPEVKFNWYVDGVEVHNAKTKPREEQYNATYRVVSVLTVLHQDWLNGKEYKCKVSNKALPAPIEKTISKAKGQPREPQVCTLPPSRDELTKNQVSLWCLVKGFYPSDIAVEWESNGQPENNYKTTPPVLDSDGSFFLYSKLTVDKSRWQQGNVFSCSVMHEALHNHYTQKSLSLSP

SEQ ID NO: 34 - protein, 444 aa, synthetic construct
  REGION 1..444: note = An artificially synthesized peptide sequence
QDQLVQSGAEVKKPGASVKVSCKASGFNIKDTYIQWVRQAPGQGLEWMGRIDPLRKQTKYREKFEGRVTITADTSTNTAYMELSSLRSEDTAVYYCVRSGREFDYWGQGTLVTVSSASTKGPSVFPLAPSSKSTSGGTAALGCLVKDYFPEPVTVSWNSGALTSGVHTFPAVLQSSGLYSLSSVVTVPSSSLGTQTYICNVNHKPSNTKVDKKVEPKSCDKTHTCPPCPAPELLGGPSVFLFPPKPKDTLMISRTPEVTCVVVDVSHEEPEVKFNWYVDGVEVHNAKTKPREEQYNSTYRVVSVLTVLHQDWLNGKEYKCKVSNDALPMPIEETISKAKGQPREPQVYTLPPSRCELTKNQVSLSCAVKGFYPSDIAVEWESNGQPENNYKTTPPVLDSDGSFFLVSKLTVDKSRWQQGNVFSCSVMHEALHNHYTQKSLSLSP

SEQ ID NO: 35 - protein, 213 aa, synthetic construct
  REGION 1..213: note = An artificially synthesized peptide sequence
DIQMTQSPSSLSASVGDRVTITCRASQDIHKYIAWYQQKPGQAPRLLIQYTSTLQPGVPSRFSGSGSGTDYTFTISSLQPEDIATYYCLQYEQLRTFGGGTKVEIKRTVAAPSVFIFPPSDEQLKSGTASVVCLLNNFYPREAKVQWKVDNALQSGNSQESVTEQDSKDSTYSLSSTLTLSKADYEKHKVYACEVTHQGLSSPVTKSFNRGEC

SEQ ID NO: 36 - protein, 22 aa, synthetic construct
  REGION 1..22: note = An artificially synthesized peptide sequence
RWGYHLRDRKYKGVRSHKGVPR

SEQ ID NO: 37 - protein, 480 aa, synthetic construct
  REGION 1..480: note = An artificially synthesized peptide sequence
EVQLVETGGSLVQPGKSLKLTCATSGFTFSNAWMHWVRQSPEKQLEWVAQIKAKRWGYHLRDRKYKGVRSHKGVPRSNNYATYYAESVKGRFTISRDDSKSNIYLQMNSLKEEDTAVYYCRYVHYGAYYGVDAWGQGTSVTVSSASTKGPSVFPLAPSSKSTSGGTAALGCLVKDYFPEPVTVSWNSGALTSGVHTFPAVLQSSGLYSLSSVVTVPSSSLGTQTYICNVNHKPSNTKVDKKVEPKSCDKTHTCPPCPAPEAAGGPSVFLFPPKPKDTLMISRTPEVTCVVVDVSHEDPEVKFNWYVDGVEVHNAKTKPREEQYASTYRVVSVLTVLHQDWLNGKEYKCKVSNKALPAPIEKTISKAKGQPREPQVYTLPPSRCELTKNQVSLSCAVKGFYPSDIAVEWESNGQPENNYKTTPPVLDSDGSFFLVSKLTVDKSRWQQGNVFSCSVMHEALHNHYTQKSLSLSPDYKDDDDK

SEQ ID NO: 38 - protein, 482 aa, synthetic construct
  REGION 1..482: note = An artificially synthesized peptide sequence
EVQLVETGGSLVQPGKSLKLTCATSGFTFSNAWMHWVRQSPEKQLEWVAQIKAKCRWGYHLRDRKYKGVRSHKGVPRCSNNYATYYAESVKGRFTISRDDSKSNIYLQMNSLKEEDTAVYYCRYVHYGAYYGVDAWGQGTSVTVSSASTKGPSVFPLAPSSKSTSGGTAALGCLVKDYFPEPVTVSWNSGALTSGVHTFPAVLQSSGLYSLSSVVTVPSSSLGTQTYICNVNHKPSNTKVDKKVEPKSCDKTHTCPPCPAPEAAGGPSVFLFPPKPKDTLMISRTPEVTCVVVDVSHEDPEVKFNWYVDGVEVHNAKTKPREEQYASTYRVVSVLTVLHQDWLNGKEYKCKVSNKALPAPIEKTISKAKGQPREPQVYTLPPSRCELTKNQVSLSCAVKGFYPSDIAVEWESNGQPENNYKTTPPVLDSDGSFFLVSKLTVDKSRWQQGNVFSCSVMHEALHNHYTQKSLSLSPDYKDDDDK

SEQ ID NO: 39 - protein, 480 aa, synthetic construct
  REGION 1..480: note = An artificially synthesized peptide sequence
EVQLVETGGSLVQPGKSLKLTCATSGFTFSNAWMHWVRQSPEKQLEWVAQIKAKSNNYATYYAESVKGRFTISRDRWGYHLRDRKYKGVRSHKGVPRDSKSNIYLQMNSLKEEDTAVYYCRYVHYGAYYGVDAWGQGTSVTVSSASTKGPSVFPLAPSSKSTSGGTAALGCLVKDYFPEPVTVSWNSGALTSGVHTFPAVLQSSGLYSLSSVVTVPSSSLGTQTYICNVNHKPSNTKVDKKVEPKSCDKTHTCPPCPAPEAAGGPSVFLFPPKPKDTLMISRTPEVTCVVVDVSHEDPEVKFNWYVDGVEVHNAKTKPREEQYASTYRVVSVLTVLHQDWLNGKEYKCKVSNKALPAPIEKTISKAKGQPREPQVYTLPPSRCELTKNQVSLSCAVKGFYPSDIAVEWESNGQPENNYKTTPPVLDSDGSFFLVSKLTVDKSRWQQGNVFSCSVMHEALHNHYTQKSLSLSPDYKDDDDK

SEQ ID NO: 40 - protein, 482 aa, synthetic construct
  REGION 1..482: note = An artificially synthesized peptide sequence
EVQLVETGGSLVQPGKSLKLTCATSGFTFSNAWMHWVRQSPEKQLEWVAQIKAKSNNYATYYAESVKGRFTISRDCRWGYHLRDRKYKGVRSHKGVPRCDSKSNIYLQMNSLKEEDTAVYYCRYVHYGAYYGVDAWGQGTSVTVSSASTKGPSVFPLAPSSKSTSGGTAALGCLVKDYFPEPVTVSWNSGALTSGVHTFPAVLQSSGLYSLSSVVTVPSSSLGTQTYICNVNHKPSNTKVDKKVEPKSCDKTHTCPPCPAPEAAGGPSVFLFPPKPKDTLMISRTPEVTCVVVDVSHEDPEVKFNWYVDGVEVHNAKTKPREEQYASTYRVVSVLTVLHQDWLNGKEYKCKVSNKALPAPIEKTISKAKGQPREPQVYTLPPSRCELTKNQVSLSCAVKGFYPSDIAVEWESNGQPENNYKTTPPVLDSDGSFFLVSKLTVDKSRWQQGNVFSCSVMHEALHNHYTQKSLSLSPDYKDDDDK

SEQ ID NO: 41 - protein, 477 aa, synthetic construct
  REGION 1..477: note = An artificially synthesized peptide sequence
EVQLVETGGSLVQPGKSLKLTCATSGFTFSNAWMHWVRQSPEKQLEWVAQIKAKSNNYATYYAESVKGRFTISRDDSKSNIYLQMNSLKEEDTAVYYCRYVHYGAYYGVDAWGQGTSVTVSSASTKGPSVFPLAPSSKSTSGGTAALGCLVKDYFPEPVTVSWNSGALTSGVHTFPAVLQSSGLYSLSSVVTVPSSSLGTQTYICNVNHKPSNTKVDKKVEPKSCDKTHTCPPCPAPELLGGPSVFLFPPKPKDTLMISRTPEVTCVVVDVSHEEPEVKFNWYVDGVEVHNAKTKPREEQYNSTYRVVSVLTVLHQDWLNGKEYKCKVSNDALPMPIEETISKAKGQPREPQVYTLPPSRCELTKNQVSLSCAVKGFYPSDIAVEWESNGQPENNYKTTPPVLDSDGSFFLVSKLTVDKSRWQQGNVFSCSVMHEALHNHYTQKSLSLSPGGGGSRWGYHLRDRKYKGVRSHKGVPR

SEQ ID NO: 42 - protein, 479 aa, synthetic construct
  REGION 1..479: note = An artificially synthesized peptide sequence
EVQLVETGGSLVQPGKSLKLTCATSGFTFSNAWMHWVRQSPEKQLEWVAQIKAKSNNYATYYAESVKGRFTISRDDSKSNIYLQMNSLKEEDTAVYYCRYVHYGAYYGVDAWGQGTSVTVSSASTKGPSVFPLAPSSKSTSGGTAALGCLVKDYFPEPVTVSWNSGALTSGVHTFPAVLQSSGLYSLSSVVTVPSSSLGTQTYICNVNHKPSNTKVDKKVEPKSCDKTHTCPPCPAPELLGGPSVFLFPPKPKDTLMISRTPEVTCVVVDVSHEEPEVKFNWYVDGVEVHNAKTKPREEQYNSTYRVVSVLTVLHQDWLNGKEYKCKVSNDALPMPIEETISKAKGQPREPQVYTLPPSRCELTKNQVSLSCAVKGFYPSDIAVEWESNGQPENNYKTTPPVLDSDGSFFLVSKLTVDKSRWQQGNVFSCSVMHEALHNHYTQKSLSLSPGGGGSCRWGYHLRDRKYKGVRSHKGVPRC

SEQ ID NO: 43 - protein, 461 aa, synthetic construct
  REGION 1..461: note = An artificially synthesized peptide sequence
EVQLVETGGSLVQPGKSLKLTCATSGFTFSNAWMHWVRQSPEKQLEWVAQIKAKGGSSNNYATYYAESVKGRFTISRDDSKSNIYLQMNSLKEEDTAVYYCRYVHYGAYYGVDAWGQGTSVTVSSASTKGPSVFPLAPSSKSTSGGTAALGCLVKDYFPEPVTVSWNSGALTSGVHTFPAVLQSSGLYSLSSVVTVPSSSLGTQTYICNVNHKPSNTKVDKKVEPKSCDKTHTCPPCPAPEAAGGPSVFLFPPKPKDTLMISRTPEVTCVVVDVSHEDPEVKFNWYVDGVEVHNAKTKPREEQYASTYRVVSVLTVLHQDWLNGKEYKCKVSNKALPAPIEKTISKAKGQPREPQVYTLPPSRCELTKNQVSLSCAVKGFYPSDIAVEWESNGQPENNYKTTPPVLDSDGSFFLVSKLTVDKSRWQQGNVFSCSVMHEALHNHYTQKSLSLSPDYKDDDDK

SEQ ID NO: 44 - protein, 464 aa, synthetic construct
  REGION 1..464: note = An artificially synthesized peptide sequence
EVQLVETGGSLVQPGKSLKLTCATSGFTFSNAWMHWVRQSPEKQLEWVAQIKAKGGSGGSSNNYATYYAESVKGRFTISRDDSKSNIYLQMNSLKEEDTAVYYCRYVHYGAYYGVDAWGQGTSVTVSSASTKGPSVFPLAPSSKSTSGGTAALGCLVKDYFPEPVTVSWNSGALTSGVHTFPAVLQSSGLYSLSSVVTVPSSSLGTQTYICNVNHKPSNTKVDKKVEPKSCDKTHTCPPCPAPEAAGGPSVFLFPPKPKDTLMISRTPEVTCVVVDVSHEDPEVKFNWYVDGVEVHNAKTKPREEQYASTYRVVSVLTVLHQDWLNGKEYKCKVSNKALPAPIEKTISKAKGQPREPQVYTLPPSRCELTKNQVSLSCAVKGFYPSDIAVEWESNGQPENNYKTTPPVLDSDGSFFLVSKLTVDKSRWQQGNVFSCSVMHEALHNHYTQKSLSLSPDYKDDDDK

SEQ ID NO: 45 - protein, 467 aa, synthetic construct
  REGION 1..467: note = An artificially synthesized peptide sequence
EVQLVETGGSLVQPGKSLKLTCATSGFTFSNAWMHWVRQSPEKQLEWVAQIKAKGGSGGSGGSSNNYATYYAESVKGRFTISRDDSKSNIYLQMNSLKEEDTAVYYCRYVHYGAYYGVDAWGQGTSVTVSSASTKGPSVFPLAPSSKSTSGGTAALGCLVKDYFPEPVTVSWNSGALTSGVHTFPAVLQSSGLYSLSSVVTVPSSSLGTQTYICNVNHKPSNTKVDKKVEPKSCDKTHTCPPCPAPEAAGGPSVFLFPPKPKDTLMISRTPEVTCVVVDVSHEDPEVKFNWYVDGVEVHNAKTKPREEQYASTYRVVSVLTVLHQDWLNGKEYKCKVSNKALPAPIEKTISKAKGQPREPQVYTLPPSRCELTKNQVSLSCAVKGFYPSDIAVEWESNGQPENNYKTTPPVLDSDGSFFLVSKLTVDKSRWQQGNVFSCSVMHEALHNHYTQKSLSLSPDYKDDDDK

SEQ ID NO: 46 - protein, 461 aa, synthetic construct
  REGION 1..461: note = An artificially synthesized peptide sequence
EVQLVETGGSLVQPGKSLKLTCATSGFTFSNAWMHWVRQSPEKQLEWVAQIKAKSNNYATYYAESVKGRFTISRDGGSDSKSNIYLQMNSLKEEDTAVYYCRYVHYGAYYGVDAWGQGTSVTVSSASTKGPSVFPLAPSSKSTSGGTAALGCLVKDYFPEPVTVSWNSGALTSGVHTFPAVLQSSGLYSLSSVVTVPSSSLGTQTYICNVNHKPSNTKVDKKVEPKSCDKTHTCPPCPAPEAAGGPSVFLFPPKPKDTLMISRTPEVTCVVVDVSHEDPEVKFNWYVDGVEVHNAKTKPREEQYASTYRVVSVLTVLHQDWLNGKEYKCKVSNKALPAPIEKTISKAKGQPREPQVYTLPPSRCELTKNQVSLSCAVKGFYPSDIAVEWESNGQPENNYKTTPPVLDSDGSFFLVSKLTVDKSRWQQGNVFSCSVMHEALHNHYTQKSLSLSPDYKDDDDK

SEQ ID NO: 47 - protein, 464 aa, synthetic construct
  REGION 1..464: note = An artificially synthesized peptide sequence
EVQLVETGGSLVQPGKSLKLTCATSGFTFSNAWMHWVRQSPEKQLEWVAQIKAKSNNYATYYAESVKGRFTISRDGGSGGSDSKSNIYLQMNSLKEEDTAVYYCRYVHYGAYYGVDAWGQGTSVTVSSASTKGPSVFPLAPSSKSTSGGTAALGCLVKDYFPEPVTVSWNSGALTSGVHTFPAVLQSSGLYSLSSVVTVPSSSLGTQTYICNVNHKPSNTKVDKKVEPKSCDKTHTCPPCPAPEAAGGPSVFLFPPKPKDTLMISRTPEVTCVVVDVSHEDPEVKFNWYVDGVEVHNAKTKPREEQYASTYRVVSVLTVLHQDWLNGKEYKCKVSNKALPAPIEKTISKAKGQPREPQVYTLPPSRCELTKNQVSLSCAVKGFYPSDIAVEWESNGQPENNYKTTPPVLDSDGSFFLVSKLTVDKSRWQQGNVFSCSVMHEALHNHYTQKSLSLSPDYKDDDDK

SEQ ID NO: 48 - protein, 467 aa, synthetic construct
  REGION 1..467: note = An artificially synthesized peptide sequence
EVQLVETGGSLVQPGKSLKLTCATSGFTFSNAWMHWVRQSPEKQLEWVAQIKAKSNNYATYYAESVKGRFTISRDGGSGGSGGSDSKSNIYLQMNSLKEEDTAVYYCRYVHYGAYYGVDAWGQGTSVTVSSASTKGPSVFPLAPSSKSTSGGTAALGCLVKDYFPEPVTVSWNSGALTSGVHTFPAVLQSSGLYSLSSVVTVPSSSLGTQTYICNVNHKPSNTKVDKKVEPKSCDKTHTCPPCPAPEAAGGPSVFLFPPKPKDTLMISRTPEVTCVVVDVSHEDPEVKFNWYVDGVEVHNAKTKPREEQYASTYRVVSVLTVLHQDWLNGKEYKCKVSNKALPAPIEKTISKAKGQPREPQVYTLPPSRCELTKNQVSLSCAVKGFYPSDIAVEWESNGQPENNYKTTPPVLDSDGSFFLVSKLTVDKSRWQQGNVFSCSVMHEALHNHYTQKSLSLSPDYKDDDDK

SEQ ID NO: 49 - protein, 461 aa, synthetic construct
  REGION 1..461: note = An artificially synthesized peptide sequence
EVQLVETGGSLVQPGKSLKLTCATSGFTFSNAWMHWVRQSPEKQLEWVAQIKAKSNNYATYYAESVKGRFTISRDDSKSNIYLQMNSLKEEDTAVYYCRYVHYGAGGSYYGVDAWGQGTSVTVSSASTKGPSVFPLAPSSKSTSGGTAALGCLVKDYFPEPVTVSWNSGALTSGVHTFPAVLQSSGLYSLSSVVTVPSSSLGTQTYICNVNHKPSNTKVDKKVEPKSCDKTHTCPPCPAPEAAGGPSVFLFPPKPKDTLMISRTPEVTCVVVDVSHEDPEVKFNWYVDGVEVHNAKTKPREEQYASTYRVVSVLTVLHQDWLNGKEYKCKVSNKALPAPIEKTISKAKGQPREPQVYTLPPSRCELTKNQVSLSCAVKGFYPSDIAVEWESNGQPENNYKTTPPVLDSDGSFFLVSKLTVDKSRWQQGNVFSCSVMHEALHNHYTQKSLSLSPDYKDDDDK

SEQ ID NO: 50 - protein, 464 aa, synthetic construct
  REGION 1..464: note = An artificially synthesized peptide sequence
EVQLVETGGSLVQPGKSLKLTCATSGFTFSNAWMHWVRQSPEKQLEWVAQIKAKSNNYATYYAESVKGRFTISRDDSKSNIYLQMNSLKEEDTAVYYCRYVHYGAGGSGGSYYGVDAWGQGTSVTVSSASTKGPSVFPLAPSSKSTSGGTAALGCLVKDYFPEPVTVSWNSGALTSGVHTFPAVLQSSGLYSLSSVVTVPSSSLGTQTYICNVNHKPSNTKVDKKVEPKSCDKTHTCPPCPAPEAAGGPSVFLFPPKPKDTLMISRTPEVTCVVVDVSHEDPEVKFNWYVDGVEVHNAKTKPREEQYASTYRVVSVLTVLHQDWLNGKEYKCKVSNKALPAPIEKTISKAKGQPREPQVYTLPPSRCELTKNQVSLSCAVKGFYPSDIAVEWESNGQPENNYKTTPPVLDSDGSFFLVSKLTVDKSRWQQGNVFSCSVMHEALHNHYTQKSLSLSPDYKDDDDK

SEQ ID NO: 51 - protein, 467 aa, synthetic construct
  REGION 1..467: note = An artificially synthesized peptide sequence
EVQLVETGGSLVQPGKSLKLTCATSGFTFSNAWMHWVRQSPEKQLEWVAQIKAKSNNYATYYAESVKGRFTISRDDSKSNIYLQMNSLKEEDTAVYYCRYVHYGAGGSGGSGGSYYGVDAWGQGTSVTVSSASTKGPSVFPLAPSSKSTSGGTAALGCLVKDYFPEPVTVSWNSGALTSGVHTFPAVLQSSGLYSLSSVVTVPSSSLGTQTYICNVNHKPSNTKVDKKVEPKSCDKTHTCPPCPAPEAAGGPSVFLFPPKPKDTLMISRTPEVTCVVVDVSHEDPEVKFNWYVDGVEVHNAKTKPREEQYASTYRVVSVLTVLHQDWLNGKEYKCKVSNKALPAPIEKTISKAKGQPREPQVYTLPPSRCELTKNQVSLSCAVKGFYPSDIAVEWESNGQPENNYKTTPPVLDSDGSFFLVSKLTVDKSRWQQGNVFSCSVMHEALHNHYTQKSLSLSPDYKDDDDK

SEQ ID NO: 52 - protein, 122 aa, synthetic construct
  REGION 1..122: note = An artificially synthesized peptide sequence
QVQLVESGGGVVQPGRSLRLSCAASGFTFSNAWMHWVRQAPGKGLEWVAQIKAKSNNYATYYAESVKGRFTISRDDSKNSLYLQMNSLKTEDTAVYYCRYVHYGAYYGVDAWGQGTTVTVSS

SEQ ID NO: 53 - protein, 112 aa, synthetic construct
  REGION 1..112: note = An artificially synthesized peptide sequence
DIVMTQSPLSLPVTPGEPASISCRSSQSLVHSNRNTYLHWYQQKPGQAPRLLIYKVSNRFSGVPDRFSGSGSGTDFTLKISRVEAEDVGVYYCGQGTQVPYTFGQGTKLEIK

SEQ ID NO: 54 - protein, 336 aa, synthetic construct
  REGION 1..336: note = An artificially synthesized peptide sequence
ASTKGPSVFPLAPSSKSTSGGTAALGCLVKDYFPEPVTVSWNSGALTSGVHTFPAVLQSSGLYSLSSVVTVPSSSLGTQTYICNVNHKPSNTKVDKKVEPKSCDKTHTCPPCPAPEAAGGPSVFLFPPKPKDTLMISRTPEVTCVVVDVSHEDPEVKFNWYVDGVEVHNAKTKPREEQYASTYRVVSVLTVLHQDWLNGKEYKCKVSNKALPAPIEKTISKAKGQPREPQVYTLPPSRCELTKNQVSLSCAVKGFYPSDIAVEWESNGQPENNYKTTPPVLDSDGSFFLVSKLTVDKSRWQQGNVFSCSVMHEALHNHYTQKSLSLSPDYKDDDDK

SEQ ID NO: 55 - protein, 107 aa, Homo sapiens [sequence omitted]

SEQ ID NO: 56 - protein, 230 aa, synthetic construct
  REGION 1..230: note = An artificially synthesized peptide sequence
EPKSSDKTHTCPPCPAPELLGGPSVFLFPPKPKDTLMISRTPEVTCVVVDVSHEDPEVKFNWYVDGVEVHNAKTKPREEQYNSTYRVVSVLTVLHQDWLNGKEYKCKVSNKALPAPIEKTISKAKGQPREPQVCTLPPSRDELTKNQVSLWCLVKGFYPSDIAVEWESNGQPENNYKTTPPVLDSDGSFFLYSKLTVDKSRWQQGNVFSCSVMHEALHNRYTQKSLSLSP

SEQ ID NO: 57 - protein, 449 aa, synthetic construct
  REGION 1..449: note = An artificially synthesized peptide sequence
QVQLQESGPGLVRPSQTLSLTCTVSGYSITSDHAWSWVRQPPGRGLEWIGYISYSGITTYNPSLKSRVTMLRDTSKNQFSLRLSSVTAADTAVYYCARSLARTTAMDYWGQGSLVTVSSASTKGPSVFPLAPSSKSTSGGTAALGCLVKDYFPEPVTVSWNSGALTSGVHTFPAVLQSSGLYSLSSVVTVPSSSLGTQTYICNVNHKPSNTKVDKKVEPKSCDKTHTCPPCPAPELLGGPSVFLFPPKPKDTLMISRTPEVTCVVVDVSHEDPEVKFNWYVDGVEVHNAKTKPREEQYNSTYRVVSVLTVLHQDWLNGKEYKCKVSNKALPAPIEKTISKAKGQPREPQVYTLPPSRDELTKNQVSLTCLVKGFYPSDIAVEWESNGQPENNYKTTPPVLDSDGSFFLYSKLTVDKSRWQQGNVFSCSVMHEALHNHYTQKSLSLSPGK

SEQ ID NO: 58 - protein, 214 aa, synthetic construct [sequence omitted]

SEQ ID NO: 59 - protein, 458 aa, synthetic construct
  REGION 1..458: note = An artificially synthesized peptide sequence
QVQLVESGGGLVQPGRSLRLSCAASGFTFSNAWMHWVRQAPGKGLEWVAQIKDKSNNYATYYAESVKGRFTISRDDSKNSIYLQMNSLKTEDTAVYYCRYVHYAAYYGVDAWGQGTTVTVSSASTKGPSVFPLAPSSKSTSGGTAALGCLVKDYFPEPVTVSWNSGALTSGVHTFPAVLQSSGLYSLSSVVTVPSSSLGTQTYICNVNHKPSNTKVDKKVEPKSCDKTHTCPPCPAPEAAGGPSVFLFPPKPKDTLMISRTPEVTCVVVDVSHEDPEVKFNWYVDGVEVHNAKTKPREEQYASTYRVVSVLTVLHQDWLNGKEYKCKVSNKALPAPIEKTISKAKGQPREPQVYTLPPSRCELTKNQVSLSCAVKGFYPSDIAVEWESNGQPENNYKTTPPVLDSDGSFFLVSKLTVDKSRWQQGNVFSCSVMHEALHNHYTQKSLSLSPDYKDDDDK

SEQ ID NO: 60 - protein, 15 aa, synthetic construct
  REGION 1..15: note = An artificially synthesized peptide sequence
QDGNEEMGGITQTPY

SEQ ID NO: 61 - protein, 467 aa, synthetic construct
  REGION 1..467: note = An artificially synthesized peptide sequence
QVQLVESGGGLVQPGRSLRLSCAASGFTFSSAWMHWVRQAPGKGLEWVAQIKDKGNGYNAYYAPSVKGRFTISRDDSKNSIYLQMNSLKTEDTAVYYCRYVHYTTSYFGLFGGGGGGVDAWGQGTTVTVSSASTKGPSVFPLAPSSKSTSGGTAALGCLVKDYFPEPVTVSWNSGALTSGVHTFPAVLQSSGLYSLSSVVTVPSSSLGTQTYICNVNHKPSNTKVDKKVEPKSCDKTHTCPPCPAPEAAGGPSVFLFPPKPKDTLMISRTPEVTCVVVDVSHEDPEVKFNWYVDGVEVHNAKTKPREEQYASTYRVVSVLTVLHQDWLNGKEYKCKVSNKALPAPIEKTISKAKGQPREPQVYTLPPSRCELTKNQVSLSCAVKGFYPSDIAVEWESNGQPENNYKTTPPVLDSDGSFFLVSKLTVDKSRWQQGNVFSCSVMHEALHNHYTQKSLSLSPDYKDDDDK

SEQ ID NO: 62 - protein, 467 aa, synthetic construct; identical to SEQ ID NO: 61
  REGION 1..467: note = An artificially synthesized peptide sequence

SEQ ID NO: 63 - protein, 464 aa, synthetic construct
  REGION 1..464: note = An artificially synthesized peptide sequence
QVQLVESGGGLVQPGRSLRLSCAASGFTFSNAWMHWVRQAPGKGLEWVAQIKDKGQQYAAYYAPSVKGRFTISRDDSKNSIYLQMNSLKTEDTAVYYCRYVHYQTYSDGSFYFGVDAWGQGTTVTVSSASTKGPSVFPLAPSSKSTSGGTAALGCLVKDYFPEPVTVSWNSGALTSGVHTFPAVLQSSGLYSLSSVVTVPSSSLGTQTYICNVNHKPSNTKVDKKVEPKSCDKTHTCPPCPAPEAAGGPSVFLFPPKPKDTLMISRTPEVTCVVVDVSHEDPEVKFNWYVDGVEVHNAKTKPREEQYASTYRVVSVLTVLHQDWLNGKEYKCKVSNKALPAPIEKTISKAKGQPREPQVYTLPPSRCELTKNQVSLSCAVKGFYPSDIAVEWESNGQPENNYKTTPPVLDSDGSFFLVSKLTVDKSRWQQGNVFSCSVMHEALHNHYTQKSLSLSPDYKDDDDK

SEQ ID NO: 64 - protein, 464 aa, synthetic construct
  REGION 1..464: note = An artificially synthesized peptide sequence
QVQLVESGGGLVQPGRSLRLSCAASGFTFSNAWMHWVRQAPGKGLEWVAQIKDRVNQYANYYAESVKGRFTISRDDSKNSIYLQMNSLKTEDTAVYYCRYVHYGLTGYFSGQGGVDAWGQGTTVTVSSASTKGPSVFPLAPSSKSTSGGTAALGCLVKDYFPEPVTVSWNSGALTSGVHTFPAVLQSSGLYSLSSVVTVPSSSLGTQTYICNVNHKPSNTKVDKKVEPKSCDKTHTCPPCPAPEAAGGPSVFLFPPKPKDTLMISRTPEVTCVVVDVSHEDPEVKFNWYVDGVEVHNAKTKPREEQYASTYRVVSVLTVLHQDWLNGKEYKCKVSNKALPAPIEKTISKAKGQPREPQVYTLPPSRCELTKNQVSLSCAVKGFYPSDIAVEWESNGQPENNYKTTPPVLDSDGSFFLVSKLTVDKSRWQQGNVFSCSVMHEALHNHYTQKSLSLSPDYKDDDDK

SEQ ID NO: 65 - protein, 464 aa, synthetic construct
  REGION 1..464: note = An artificially synthesized peptide sequence
QVQLVESGGGLVQPGRSLRLSCAASGFTFSNAWMHWVRQAPGKGLEWVAQIKDRVNQYANYYAESVKGRLTISRDDSKNSIYLQMNSLKTEDTAVYYCRYVHYGLTGYFSGQGGVDAWGQGTTVTVSSASTKGPSVFPLAPSSKSTSGGTAALGCLVKDYFPEPVTVSWNSGALTSGVHTFPAVLQSSGLYSLSSVVTVPSSSLGTQTYICNVNHKPSNTKVDKKVEPKSCDKTHTCPPCPAPEAAGGPSVFLFPPKPKDTLMISRTPEVTCVVVDVSHEDPEVKFNWYVDGVEVHNAKTKPREEQYASTYRVVSVLTVLHQDWLNGKEYKCKVSNKALPAPIEKTISKAKGQPREPQVYTLPPSRCELTKNQVSLSCAVKGFYPSDIAVEWESNGQPENNYKTTPPVLDSDGSFFLVSKLTVDKSRWQQGNVFSCSVMHEALHNHYTQKSLSLSPDYKDDDDK

SEQ ID NO: 66 - protein, 464 aa, synthetic construct
  REGION 1..464: note = An artificially synthesized peptide sequence
QVQLVESGGGLVQPGRSLRLSCAASGFAFSNAWMHWVRQAPGKGLEWVAQIKDRVNQYANYYAESVKGRFTISRDDSKNSIYLQMNSLKTEDTAVYYCRYVHYGLTGYFSGQGGVDAWGQGTTVTVSSASTKGPSVFPLAPSSKSTSGGTAALGCLVKDYFPEPVTVSWNSGALTSGVHTFPAVLQSSGLYSLSSVVTVPSSSLGTQTYICNVNHKPSNTKVDKKVEPKSCDKTHTCPPCPAPEAAGGPSVFLFPPKPKDTLMISRTPEVTCVVVDVSHEDPEVKFNWYVDGVEVHNAKTKPREEQYASTYRVVSVLTVLHQDWLNGKEYKCKVSNKALPAPIEKTISKAKGQPREPQVYTLPPSRCELTKNQVSLSCAVKGFYPSDIAVEWESNGQPENNYKTTPPVLDSDGSFFLVSKLTVDKSRWQQGNVFSCSVMHEALHNHYTQKSLSLSPDYKDDDDK

SEQ ID NO: 67 - protein, 464 aa, synthetic construct
  REGION 1..464: note = An artificially synthesized peptide sequence
QVQLVESGGGLVQPGRSLRLSCAASGFTFSNAWMHWVRQAPGKGLEWVAQIKDRVNQYANYYAECVKGRFTISRDDSKNSIYLQMNSLKTEDTAVYYCRYVHYGLTGYFSGQGGVDAWGQGTTVTVSSASTKGPSVFPLAPSSKSTSGGTAALGCLVKDYFPEPVTVSWNSGALTSGVHTFPAVLQSSGLYSLSSVVTVPSSSLGTQTYICNVNHKPSNTKVDKKVEPKSCDKTHTCPPCPAPEAAGGPSVFLFPPKPKDTLMISRTPEVTCVVVDVSHEDPEVKFNWYVDGVEVHNAKTKPREEQYASTYRVVSVLTVLHQDWLNGKEYKCKVSNKALPAPIEKTISKAKGQPREPQVYTLPPSRCELTKNQVSLSCAVKGFYPSDIAVEWESNGQPENNYKTTPPVLDSDGSFFLVSKLTVDKSRWQQGNVFSCSVMHEALHNHYTQKSLSLSPDYKDDDDK

SEQ ID NO: 68 - protein, 464 aa, synthetic construct
  REGION 1..464: note = An artificially synthesized peptide sequence
QVQLVESGGGLVQPGRSLRLSCAASGFTFSSAWMHWVRQAPGKGLEWVAQIKDKQNQYNAYYAESVKGRFTISRDDSKNSIYLQMNSLKTEDTAVYYCRYVHYATSDGFLPYFGVDAWGQGTTVTVSSASTKGPSVFPLAPSSKSTSGGTAALGCLVKDYFPEPVTVSWNSGALTSGVHTFPAVLQSSGLYSLSSVVTVPSSSLGTQTYICNVNHKPSNTKVDKKVEPKSCDKTHTCPPCPAPEAAGGPSVFLFPPKPKDTLMISRTPEVTCVVVDVSHEDPEVKFNWYVDGVEVHNAKTKPREEQYASTYRVVSVLTVLHQDWLNGKEYKCKVSNKALPAPIEKTISKAKGQPREPQVYTLPPSRCELTKNQVSLSCAVKGFYPSDIAVEWESNGQPENNYKTTPPVLDSDGSFFLVSKLTVDKSRWQQGNVFSCSVMHEALHNHYTQKSLSLSPDYKDDDDK

SEQ ID NO: 69 - protein, 464 aa, synthetic construct
  REGION 1..464: note = An artificially synthesized peptide sequence
QVQLVESGGGLVQPGRSLRLSCAASGFTFSNAWMHWVRQAPGKGLEWVAQIKDRASGYNNYYAESVKGRFTISRDDSKNSIYLQMNSLKTEDTAVYYCRYVHYAQSVSAFFQYGVDAWGQGTTVTVSSASTKGPSVFPLAPSSKSTSGGTAALGCLVKDYFPEPVTVSWNSGALTSGVHTFPAVLQSSGLYSLSSVVTVPSSSLGTQTYICNVNHKPSNTKVDKKVEPKSCDKTHTCPPCPAPEAAGGPSVFLFPPKPKDTLMISRTPEVTCVVVDVSHEDPEVKFNWYVDGVEVHNAKTKPREEQYASTYRVVSVLTVLHQDWLNGKEYKCKVSNKALPAPIEKTISKAKGQPREPQVYTLPPSRCELTKNQVSLSCAVKGFYPSDIAVEWESNGQPENNYKTTPPVLDSDGSFFLVSKLTVDKSRWQQGNVFSCSVMHEALHNHYTQKSLSLSPDYKDDDDK

SEQ ID NO: 70 - protein, 464 aa, synthetic construct
  REGION 1..464: note = An artificially synthesized peptide sequence
QVQLVESGGGLVQPGRSLRLSCAASGFTFSNAWMHWVRQAPGKGLEWVAQIKDKQSQYANYYAPSVKGRFTISRDDSKNSIYLQMNSLKTEDTAVYYCRYVHYQSTSYSFYQGGVDAWGQGTTVTVSSASTKGPSVFPLAPSSKSTSGGTAALGCLVKDYFPEPVTVSWNSGALTSGVHTFPAVLQSSGLYSLSSVVTVPSSSLGTQTYICNVNHKPSNTKVDKKVEPKSCDKTHTCPPCPAPEAAGGPSVFLFPPKPKDTLMISRTPEVTCVVVDVSHEDPEVKFNWYVDGVEVHNAKTKPREEQYASTYRVVSVLTVLHQDWLNGKEYKCKVSNKALPAPIEKTISKAKGQPREPQVYTLPPSRCELTKNQVSLSCAVKGFYPSDIAVEWESNGQPENNYKTTPPVLDSDGSFFLVSKLTVDKSRWQQGNVFSCSVMHEALHNHYTQKSLSLSPDYKDDDDK

SEQ ID NO: 71 - protein, 464 aa, synthetic construct
  REGION 1..464: note = An artificially synthesized peptide sequence
QVQLVESGGGLVQPGRSLRLSCAASGFTFSNAWMHWVRQAPGKGLEWVAQIKDKQSQYANYYAPSVKGRFTISRDDSKSSIYLQMNSLKTEDTAVYYCRYVHYQSTSYSFYQGGVDAWGQGTTVTVSSASTKGPSVFPLAPSSKSTSGGTAALGCLVKDYFPEPVTVSWNSGALTSGVHTFPAVLQSSGLYSLSSVVTVPSSSLGTQTYICNVNHKPSNTKVDKKVEPKSCDKTHTCPPCPAPEAAGGPSVFLFPPKPKDTLMISRTPEVTCVVVDVSHEDPEVKFNWYVDGVEVHNAKTKPREEQYASTYRVVSVLTVLHQDWLNGKEYKCKVSNKALPAPIEKTISKAKGQPREPQVYTLPPSRCELTKNQVSLSCAVKGFYPSDIAVEWESNGQPENNYKTTPPVLDSDGSFFLVSKLTVDKSRWQQGNVFSCSVMHEALHNHYTQKSLSLSPDYKDDDDK

SEQ ID NO: 72 - protein, 464 aa, synthetic construct
  REGION 1..464: note = An artificially synthesized peptide sequence
QVQLVESGGGLVQPGRSLRLSCAASGFTFSNAWMHWVRQAPGKGLEWVAQIKDRGNNYAAYYAESVKGRFTISRDDSKNSIYLQMNSLKTEDTAVYYCRYVHYGSYFFASFYFGVDIWGQGTTVTVSSASTKGPSVFPLAPSSKSTSGGTAALGCLVKDYFPEPVTVSWNSGALTSGVHTFPAVLQSSGLYSLSSVVTVPSSSLGTQTYICNVNHKPSNTKVDKKVEPKSCDKTHTCPPCPAPEAAGGPSVFLFPPKPKDTLMISRTPEVTCVVVDVSHEDPEVKFNWYVDGVEVHNAKTKPREEQYASTYRVVSVLTVLHQDWLNGKEYKCKVSNKALPAPIEKTISKAKGQPREPQVYTLPPSRCELTKNQVSLSCAVKGFYPSDIAVEWESNGQPENNYKTTPPVLDSDGSFFLVSKLTVDKSRWQQGNVFSCSVMHEALHNHYTQKSLSLSPDYKDDDDK

SEQ ID NO: 73 - protein, 464 aa, synthetic construct
  REGION 1..464: note = An artificially synthesized peptide sequence
QVQLVESGGGLVQPGHSLRLSCAASGFTFSNAWMHWVRQAPGKGLEWVAQIKDRGNNYAAYYAESVKGRFTISRDDSKNSIYLQMNSLKTEDTAVYYCRYVHYGSYFFASFYFGVDIWGQGTTVTVSSASTKGPSVFPLAPSSKSTSGGTAALGCLVKDYFPEPVTVSWNSGALTSGVHTFPAVLQSSGLYSLSSVVTVPSSSLGTQTYICNVNHKPSNTKVDKKVEPKSCDKTHTCPPCPAPEAAGGPSVFLFPPKPKDTLMISRTPEVTCVVVDVSHEDPEVKFNWYVDGVEVHNAKTKPREEQYASTYRVVSVLTVLHQDWLNGKEYKCKVSNKALPAPIEKTISKAKGQPREPQVYTLPPSRCELTKNQVSLSCAVKGFYPSDIAVEWESNGQPENNYKTTPPVLDSDGSFFLVSKLTVDKSRWQQGNVFSCSVMHEALHNHYTQKSLSLSPDYKDDDDK

SEQ ID NO: 74 - protein, 464 aa, synthetic construct
  REGION 1..464: note = An artificially synthesized peptide sequence
QVQLVESGGGLVQPGRSLRLSCAASGFTFSNAWMHWVRQAPGKGLEWVAQIKDRGNNYNTYYAPSVKGRFTISRDDSKNSIYLQMNSLKTEDTAVYYCRYVHYGSYFFSGSSFGVDIWGQGTTVTVSSASTKGPSVFPLAPSSKSTSGGTAALGCLVKDYFPEPVTVSWNSGALTSGVHTFPAVLQSSGLYSLSSVVTVPSSSLGTQTYICNVNHKPSNTKVDKKVEPKSCDKTHTCPPCPAPEAAGGPSVFLFPPKPKDTLMISRTPEVTCVVVDVSHEDPEVKFNWYVDGVEVHNAKTKPREEQYASTYRVVSVLTVLHQDWLNGKEYKCKVSNKALPAPIEKTISKAKGQPREPQVYTLPPSRCELTKNQVSLSCAVKGFYPSDIAVEWESNGQPENNYKTTPPVLDSDGSFFLVSKLTVDKSRWQQGNVFSCSVMHEALHNHYTQKSLSLSPDYKDDDDK

SEQ ID NO: 75 - protein, 464 aa, synthetic construct
  REGION 1..464: note = An artificially synthesized peptide sequence
QVQLVESGGGLVQPGRSLRLSCAASGFTFSNAWMHWVRQAPGKGLEWVAQIKDRGNNYNTYYAPSVKGRFTISRDDSKNSIYLQMNSLKTEDTAVYYCRYAHYGSYFFSGSSFGVDIWGQGTTVTVSSASTKGPSVFPLAPSSKSTSGGTAALGCLVKDYFPEPVTVSWNSGALTSGVHTFPAVLQSSGLYSLSSVVTVPSSSLGTQTYICNVNHKPSNTKVDKKVEPKSCDKTHTCPPCPAPEAAGGPSVFLFPPKPKDTLMISRTPEVTCVVVDVSHEDPEVKFNWYVDGVEVHNAKTKPREEQYASTYRVVSVLTVLHQDWLNGKEYKCKVSNKALPAPIEKTISKAKGQPREPQVYTLPPSRCELTKNQVSLSCAVKGFYPSDIAVEWESNGQPENNYKTTPPVLDSDGSFFLVSKLTVDKSRWQQGNVFSCSVMHEALHNHYTQKSLSLSPDYKDDDDK

SEQ ID NO: 76 - protein, 464 aa, synthetic construct
  REGION 1..464: note = An artificially synthesized peptide sequence
QVQLVESGGGLVQPGRSLRLSCAASGFTFSNAWMHWVRQAPGKGLEWVAQIKDKGNQYATYYAESVKGRFTISRDDSKNSIYLQMNSLKTEDTAVYYCRYVHYGTYFFALPAFGVDIWGQGTTVTVSSASTKGPSVFPLAPSSKSTSGGTAALGCLVKDYFPEPVTVSWNSGALTSGVHTFPAVLQSSGLYSLSSVVTVPSSSLGTQTYICNVNHKPSNTKVDKKVEPKSCDKTHTCPPCPAPEAAGGPSVFLFPPKPKDTLMISRTPEVTCVVVDVSHEDPEVKFNWYVDGVEVHNAKTKPREEQYASTYRVVSVLTVLHQDWLNGKEYKCKVSNKALPAPIEKTISKAKGQPREPQVYTLPPSRCELTKNQVSLSCAVKGFYPSDIAVEWESNGQPENNYKTTPPVLDSDGSFFLVSKLTVDKSRWQQGNVFSCSVMHEALHNHYTQKSLSLSPDYKDDDDK

SEQ ID NO: 77 - protein, 464 aa, synthetic construct
  REGION 1..464: note = An artificially synthesized peptide sequence
QVQLVESGGGLVQPGRSLRLSCAASGFTFSNAWMHWVRQAPGKGLEWVAQIKDKGNQYATYYAESVKGRYTISRDDSKNSIYLQMNSLKTEDTAVYYCRYVHYGTYFFALPAFGVDIWGQGTTVTVSSASTKGPSVFPLAPSSKSTSGGTAALGCLVKDYFPEPVTVSWNSGALTSGVHTFPAVLQSSGLYSLSSVVTVPSSSLGTQTYICNVNHKPSNTKVDKKVEPKSCDKTHTCPPCPAPEAAGGPSVFLFPPKPKDTLMISRTPEVTCVVVDVSHEDPEVKFNWYVDGVEVHNAKTKPREEQYASTYRVVSVLTVLHQDWLNGKEYKCKVSNKALPAPIEKTISKAKGQPREPQVYTLPPSRCELTKNQVSLSCAVKGFYPSDIAVEWESNGQPENNYKTTPPVLDSDGSFFLVSKLTVDKSRWQQGNVFSCSVMHEALHNHYTQKSLSLSPDYKDDDDK

SEQ ID NO: 78 - protein, 464 aa, synthetic construct
  REGION 1..464: note = An artificially synthesized peptide sequence
QVQLVESGGGLVQPGRSLRLSCAASGFTFSNAWMHWVRQAPGKGLEWVAQIKDRGNNYAAYYAESVKGRFTISRDDSKNSIYLQMNSLKTEDTAVYYCRYVHYGSYFFASFYFGVDIWGQGTAVTVSSASTKGPSVFPLAPSSKSTSGGTAALGCLVKDYFPEPVTVSWNSGALTSGVHTFPAVLQSSGLYSLSSVVTVPSSSLGTQTYICNVNHKPSNTKVDKKVEPKSCDKTHTCPPCPAPEAAGGPSVFLFPPKPKDTLMISRTPEVTCVVVDVSHEDPEVKFNWYVDGVEVHNAKTKPREEQYASTYRVVSVLTVLHQDWLNGKEYKCKVSNKALPAPIEKTISKAKGQPREPQVYTLPPSRCELTKNQVSLSCAVKGFYPSDIAVEWESNGQPENNYKTTPPVLDSDGSFFLVSKLTVDKSRWQQGNVFSCSVMHEALHNHYTQKSLSLSPDYKDDDDK

SEQ ID NO: 79 - protein, 15 aa, synthetic construct
  REGION 1..15: note = An artificially synthesized peptide sequence
GLNDIFEAQKIEWHE

SEQ ID NO: 80 - protein, 233 aa, synthetic construct
  REGION 1..233: note = An artificially synthesized peptide sequence
CHPRLSLHRPALEDLLLGSEANLTCTLTGLRDASGVTFTWTPSSGKSAVQGPPERDLCGCYSVSSVLPGCAEPWNHGKTFTCTAAYPESKTPLTATLSKSGNTFRPEVHLLPPPSEELALNELVTLTCLARGFSPKDVLVRWLQGSQELPREKYLTWASRQEPSQGTTTFAVTSILRVAAEDWKKGDTFSCMVGHEALPLAFTQKTIDRLAGKGGGGSGLNDIFEAQKIEWHE

SEQ ID NO: 81 - protein, 641 aa, Human herpesvirus 4
MSDEGPGTGPGNGLGEKGDTSGPEGSGGSGPQRRGGDNHGRGRGRGRGRGGGRPGAPGGSGSGPRHRDGVRRPQKRPSCIGCKGTHGGTGAGAGAGGAGAGGAGAGGGAGAGGGAGGAGGAGGAGAGGGAGAGGGAGGAGGAGAGGGAGAGGGAGGAGAGGGAGGAGGAGAGGGAGAGGGAGGAGAGGGAGGAGGAGAGGGAGAGGAGGAGGAGAGGAGAGGGAGGAGGAGAGGAGAGGAGAGGAGAGGAGGAGAGGAGGAGAGGAGGAGAGGGAGGAGAGGGAGGAGAGGAGGAGAGGAGGAGAGGAGGAGAGGGAGAGGAGAGGGGRGRGGSGGRGRGGSGGRGRGGSGGRRGRGRERARGGSRERARGRGRGRGEKRPRSPSSQSSSSGSPPRRPPPGRRPFFHPVGEADYFEYHQEGGPDGEPDVPPGAIEQGPADDPGEGPSTGPRGQGDGGRRKKGGWFGKHRGQGGSNPKFENIAEGLRALLARSHVERTTDEGTWVAGVFVYGGSKTSLYNLRRGTALAIPQCRLTPLSRLPFGMAPGPGPQPGPLRESIVCYFMVFLQTHIFAEVLKDAIKDLVMTKPAPTCNIRVTVCSFDDGVDLPPWFPPMVEGAAAEGDDGDDGDEGGDGDEGEEGQE

SEQ ID NO: 82 - protein, 321 aa, Escherichia coli
MKDNTVPLKLIALLANGEFHSGEQLGETLGMSRAAINKHIQTLRDWGVDVFTVPGKGYSLPEPIQLLNAKQILGQLDGGSVAVLPVIDSTNQYLLDRIGELKSGDACIAEYQQAGRGRRGRKWFSPFGANLYLSMFWRLEQGPAAAIGLSLVIGIVMAEVLRKLGADKVRVKWPNDLYLQDRKLAGILVELTGKTGDAAQIVIGAGINMAMRRVEESVVNQGWITLQEAGINLDRNTLAAMLIRELRAALELFEQEGLAPYLSRWEKLDNFINRPVKLIIGDKEIFGISRGIDKQGALLLEQDGIIKPWMGGEISLRSAEK

SEQ ID NO: 83 - DNA, 549 bp, Homo sapiens
  source 1..549: mol_type = unassigned DNA
atggaacaggggaagggcctggctgtcctcatcctggctatcattcttcttcaaggtactttggcccagtcaatcaaaggaaaccacttggttaaggtgtatgactatcaagaagatggttcggtacttctgacttgtgatgcagaagccaaaaatatcacatggtttaaagatgggaagatgatcggcttcctaactgaagataaaaaaaaatggaatctgggaagtaatgccaaggaccctcgagggatgtatcagtgtaaaggatcacagaacaagtcaaaaccactccaagtgtattacagaatgtgtcagaactgcattgaactaaatgcagccaccatatctggctttctctttgctgaaatcgtcagcattttcgtccttgctgttggggtctacttcattgctggacaggatggagttcgccagtcgagagcttcagacaagcagactctgttgcccaatgaccagctctaccagcccctcaaggatcgagaagatgaccagtacagccaccttcaaggaaaccagttgaggaggaattga

SEQ ID NO: 84 - protein, 182 aa, Homo sapiens
MEQGKGLAVLILAIILLQGTLAQSIKGNHLVKVYDYQEDGSVLLTCDAEAKNITWFKDGKMIGFLTEDKKKWNLGSNAKDPRGMYQCKGSQNKSKPLQVYYRMCQNCIELNAATISGFLFAEIVSIFVLAVGVYFIAGQDGVRQSRASDKQTLLPNDQLYQPLKDREDDQYSHLQGNQLRRN

SEQ ID NO: 85 - DNA, 516 bp, Homo sapiens
  source 1..516: mol_type = unassigned DNA
atggaacatagcacgtttctctctggcctggtactggctacccttctctcgcaagtgagccccttcaagatacctatagaggaacttgaggacagagtgtttgtgaattgcaataccagcatcacatgggtagagggaacggtgggaacactgctctcagacattacaagactggacctgggaaaacgcatcctggacccacgaggaatatataggtgtaatgggacagatatatacaaggacaaagaatctaccgtgcaagttcattatcgaatgtgccagagctgtgtggagctggatccagccaccgtggctggcatcattgtcactgatgtcattgccactctgctccttgctttgggagtcttctgctttgctggacatgagactggaaggctgtctggggctgccgacacacaagctctgttgaggaatgaccaggtctatcagcccctccgagatcgagatgatgctcagtacagccaccttggaggaaactgggctcggaacaagtga

SEQ ID NO: 86 - protein, 171 aa, Homo sapiens
MEHSTFLSGLVLATLLSQVSPFKIPIEELEDRVFVNCNTSITWVEGTVGTLLSDITRLDLGKRILDPRGIYRCNGTDIYKDKESTVQVHYRMCQSCVELDPATVAGIIVTDVIATLLLALGVFCFAGHETGRLSGAADTQALLRNDQVYQPLRDRDDAQYSHLGGNWARNK

SEQ ID NO: 87 - DNA, 624 bp, Homo sapiens
  source 1..624: mol_type = unassigned DNA
atgcagtcgggcactcactggagagttctgggcctctgcctcttatcagttggcgtttgggggcaagatggtaatgaagaaatgggtggtattacacagacaccatataaagtctccatctctggaaccacagtaatattgacatgccctcagtatcctggatctgaaatactatggcaacacaatgataaaaacataggcggtgatgaggatgataaaaacataggcagtgatgaggatcacctgtcactgaaggaattttcagaattggagcaaagtggttattatgtctgctaccccagaggaagcaaaccagaagatgcgaacttttatctctacctgagggcaagagtgtgtgagaactgcatggagatggatgtgatgtcggtggccacaattgtcatagtggacatctgcatcactgggggcttgctgctgctggtttactactggagcaagaatagaaaggccaaggccaagcctgtgacacgaggagcgggtgctggcggcaggcaaaggggacaaaacaaggagaggccaccacctgttcccaacccagactatgagcccatccggaaaggccagcgggacctgtattctggcctgaatcagagacgcatctga

SEQ ID NO: 88 - protein, 207 aa, Homo sapiens
MQSGTHWRVLGLCLLSVGVWGQDGNEEMGGITQTPYKVSISGTTVILTCPQYPGSEILWQHNDKNIGGDEDDKNIGSDEDHLSLKEFSELEQSGYYVCYPRGSKPEDANFYLYLRARVCENCMEMDVMSVATIVIVDICITGGLLLLVYYWSKNRKAKAKPVTRGAGAGGRQRGQNKERPPPVPNPDYEPIRKGQRDLYSGLNQRRI

SEQ ID NO: 89 - protein, 8 aa, synthetic construct
  REGION 1..8: note = An artificially synthesized peptide sequence
DYKDDDDK

SEQ ID NO: 90 - protein, 6 aa, synthetic construct
  REGION 1..6: note = An artificially synthesized peptide sequence
GGSGGS

SEQ ID NO: 91 - protein, 9 aa, synthetic construct
  REGION 1..9: note = An artificially synthesized peptide sequence
GGSGGSGGS

SEQ ID NO: 92 - protein, 7 aa, synthetic construct
  REGION 1..7: note = An artificially synthesized peptide sequence
GGSGGGS

SEQ ID NO: 93 - protein, 8 aa, synthetic construct
  REGION 1..8: note = An artificially synthesized peptide sequence
GGGSGGGS

SEQ ID NO: 94 - protein, 122 aa, synthetic construct
  REGION 1..122: note = An artificially synthesized peptide sequence
QVQLVESGGGLVQPGRSLRLSCAASGFTFSNAWMHWVRQAPGKGLEWVAQIKAKSNNYATYYAESVKGRFTISRDDSKNSIYLQMNSLKTEDTAVYYCRYVHYGAYYGVDAWGQGTTVTVSS

SEQ ID NO: 95 - protein, 122 aa, synthetic construct
  REGION 1..122: note = An artificially synthesized peptide sequence
QVQLVESGGGLVQPGRSLRLSCAASGFTFSNAWMHWVRQAPGKGLEWVAQIKDKSNNYATYYAESVKGRFTISRDDSKNSIYLQMNSLKTEDTAVYYCRYVHYGAYYGVDAWGQGTTVTVSS

SEQ ID NO: 96 - protein, 128 aa, synthetic construct
  REGION 1..128: note = An artificially synthesized peptide sequence
QVQLVESGGGLVQPGRSLRLSCAASGFTFSNAWMHWVRQAPGKGLEWVAQIKDKSNNYATYYAESVKGRFTISRDDSKNSIYLQMNSLKTEDTAVYYCRYVHYGAGGSGGSYYGVDAWGQGTTVTVSS

SEQ ID NO: 97 - protein, 122 aa, synthetic construct; identical to SEQ ID NO: 13
  REGION 1..122: note = An artificially synthesized peptide sequence

SEQ ID NO: 98 - protein, 112 aa, synthetic construct; identical to SEQ ID NO: 14
  REGION 1..112: note = An artificially synthesized peptide sequence

SEQ ID NO: 99 - protein, 5 aa, synthetic construct
  REGION 1..5: note = An artificially synthesized peptide sequence
NAWMH

SEQ ID NO: 100 - protein, 19 aa, synthetic construct
  REGION 1..19: note = An artificially synthesized peptide sequence
QIKDKSNNYATYYAESVKG

SEQ ID NO: 101 - protein, 11 aa, synthetic construct
  REGION 1..11: note = An artificially synthesized peptide sequence
VHYGAYYGVDA

SEQ ID NO: 102 - protein, 17 aa, synthetic construct
  REGION 1..17: note = An artificially synthesized peptide sequence
VHYGAGGSGGSYYGVDA

SEQ ID NO: 103 - protein, 16 aa, synthetic construct
  REGION 1..16: note = An artificially synthesized peptide sequence
RSSQSLVHSNRNTYLH

SEQ ID NO: 104 - protein, 7 aa, synthetic construct
  REGION 1..7: note = An artificially synthesized peptide sequence
KVSNRFS

SEQ ID NO: 105 - protein, 9 aa, synthetic construct
  REGION 1..9: note = An artificially synthesized peptide sequence
GQGTQVPYT

SEQ ID NO: 106 - protein, 128 aa, synthetic construct
  REGION 1..128: note = An artificially synthesized peptide sequence
QVQLVESGGGLVQPGRSLRLSCAASGFTFSNAWMHWVRQAPGKGLEWVAQIKDKANGYNTYYAPSVKGRFTISRDDSKNSIYLQMNSLKTEDTAVYYCRYVHYTTYYYASGSYGVDAWGQGTTVTVSS

SEQ ID NO: 107 - protein, 128 aa, synthetic construct
  REGION 1..128: note = An artificially synthesized peptide sequence
QVQLVESGGGLVQPGRSLRLSCAASGFTFSNAWMHWVRQAPGKGLEWVAQIKDRSNGYATYYAESVKGRFTISRDDSKNSIYLQMNSLKTEDTAVYYCRYVHYTTFTGVSFQYGVDAWGQGTTVTVSS

SEQ ID NO: 108 - protein, 128 aa, synthetic construct
  REGION 1..128: note = An artificially synthesized peptide sequence
QVQLVESGGGLVQPGRSLRLSCAASGFTFSNAWMHWVRQAPGKGLEWVAQIKDRASGYATYYAPSVKGRFTISRDDSKNSIYLQMNSLKTEDTAVYYCRYVHYTTYVDGLYSFGVDAWGQGTTVTVSS

SEQ ID NO: 109 - protein, 128 aa, synthetic construct
  REGION 1..128: note = An artificially synthesized peptide sequence
QVQLVESGGGLVQPGRSLRLSCAASGFTFSNAWMHWVRQAPGKGLEWVAQIKDKANGYNTYYAPSVKGRFTISRDDSKNSIYLQMNSLKTEDTAVYYCRYVHYTLYFGGYYQYGVDAWGQGTTVTVSS

SEQ ID NO: 110 - protein, 128 aa, synthetic construct
  REGION 1..128: note = An artificially synthesized peptide sequence
QVQLVESGGGLVQPGRSLRLSCAASGFTFSNAWMHWVRQAPGKGLEWVAQIKDKANGYNTYYAESVKGRFTISRDDSKNSIYLQMNSLKTEDTAVYYCRYVHYTTFGGFGFSYGVDAWGQGTTVTVSS

SEQ ID NO: 111 - protein, 128 aa, synthetic construct
  REGION 1..128: note = An artificially synthesized peptide sequence
QVQLVESGGGLVQPGRSLRLSCAASGFTFSNAWMHWVRQAPGKGLEWVAQIKDRQNGYNTYYAESVKGRFTISRDDSKNSIYLQMNSLKTEDTAVYYCRYVHYTTTYGSYYQFGVDAWGQGTTVTVSS

SEQ ID NO: 112 - protein, 128 aa, synthetic construct
  REGION 1..128: note = An artificially synthesized peptide sequence
QVQLVESGGGLVQPGRSLRLSCAASGFTFSNAWMHWVRQAPGKGLEWVAQIKDRQNGYAAYYAESVKGRFTISRDDSKNSIYLQMNSLKTEDTAVYYCRYVHYRTFTGLSPKFGVDAWGQGTPVTVSS

SEQ ID NO: 113 - protein, 128 aa, synthetic construct
  REGION 1..128: note = An artificially synthesized peptide sequence
QVQLVESGGGLVQPGRSLRLSCAASGFTFSNAWMHWVRQAPGKGLEWVAQIKDKQNSYAAYYAESVKGRFTISRDDSKNSIYLQMNSLKTEDTAVYYCRYVHYTTYSGGFFSYGVDAWGQGTTVTVSS

SEQ ID NO: 114 - protein, 128 aa, synthetic construct
  REGION 1..128: note = An artificially synthesized peptide sequence
QVQLVESGGGLVQPGRSLRLSCAASGFTFSNAWMHWVRQAPGKGLEWVAQIKDRANSYNTYYAESVKGRFTISRDDSKNSIYLQMNSLKTEDTAVYYCRYVHYTTYAGSSFSYGVDAWGQGTTVTVSS

SEQ ID NO: 115 - protein, 128 aa, synthetic construct
  REGION 1..128: note = An artificially synthesized peptide sequence
QVQLVESGGGLVQPGRSLRLSCAASGFTFSNAWMHWVRQAPGKGLEWVAQIKDKANGYNAYYAESVKGRFTISRDDSKNSIYLQMNSLKTEDTAVYYCRYVHYTTYAGFSYKFGVDAWGQGTTVTVSS

SEQ ID NO: 116 - protein, 128 aa, synthetic construct
  REGION 1..128: note = An artificially synthesized peptide sequence
QVQLVESGGGLVQPGRSLRLSCAASGFTFSNAWMHWVRQAPGKGLEWVAQIKDRGNGYNTYYAESVKGRFTISRDDSKNSIYLQMNSLKTEDTAVYYCRYVHYTTFGDGFYKFGVDAWGQGTTVTVSS

SEQ ID NO: 117 - protein, 126 aa, synthetic construct
  REGION 1..126: note = An artificially synthesized peptide sequence
QVQLVESGGGLVQPGRSLRLSCAASGFTFSNAWMHWVRQAPGKGLEWVAQIKDRSNGYAAYYAPSVKGRFTISRDDSKNSIYLQMNSLKTEDTAVYYCRYVHYTTFLSFAYGVDAWGQGTTVTVSS

SEQ ID NO: 118 - protein, 128 aa, synthetic construct
  REGION 1..128: note = An artificially synthesized peptide sequence
QVQLVESGGGLVQPGRSLRLSCAASGFTFSNAWMHWVRQAPGKGLEWVAQIKDRGNGYNTYYAPSVKGRFTISRDDSKNSIYLQMNSLKTEDTAVYYCRYVHYRTSSYGGFKFGVDAWGQGTTVTVSS

SEQ ID NO: 119 - protein, 128 aa, synthetic construct
  REGION 1..128: note = An artificially synthesized peptide sequence
QVQLVESGGGLVQPGRSLRLSCAASGFTFSNAWMHWVRQAPGKGLEWVAQIKDRSNGYATYYAESVKGRFTISRDDSKNSIYLQMNSLKTEDTAVYYCRYVHYTSFAFFFGQFGVDAWGQGTTVTVSS

SEQ ID NO: 120 - protein, 126 aa, synthetic construct
  REGION 1..126: note = An artificially synthesized peptide sequence
QVQLVESGGGLVQPGRSLRLSCAASGFTFSNAWMHWVRQAPGKGLEWVAQIKDKGNQYNTYYAESVKGRFTISRDDSKNSIYLQMNSLKTEDTAVYYCRYVHYTQYSFGQYGVDAWGQGTTVTVSS

SEQ ID NO: 121 - protein, 128 aa, synthetic construct
  REGION 1..128: note = An artificially synthesized peptide sequence
QVQLVESGGGLVQPGRSLRLSCAASGFTFSNAWMHWVRQAPGKGLEWVAQIKDKGNQYNAYYAPSVKGRFTISRDDSKNSIYLQMNSLKTEDTAVYYCRYVHYVSSSSGSYQFGVDAWGQGTTVTVSS

SEQ ID NO: 122 - protein, 128 aa, synthetic construct
  REGION 1..128: note = An artificially synthesized peptide sequence
QVQLVESGGGLVQPGRSLRLSCAASGFTFSNAWMHWVRQAPGKGLEWVAQIKDRGSAYAAYYAESVKGRFTISRDDSKNSIYLQMNSLKTEDTAVYYCRYVHYTSGYFGYFQYGVDAWGQGTTVTVSS

SEQ ID NO: 123 - protein, 128 aa, synthetic construct
  REGION 1..128: note = An artificially synthesized peptide sequence
QVQLVESGGGLVQPGRSLRLSCAASGFTFSNAWMHWVRQAPGKGLEWVAQIKDRGNNYLTYYAPSVKGRFTISRDDSKNSIYLQMNSLKTEDTAVYYCRYVHYTTYYGGFYSFGVDAWGQGTTVTVSS

SEQ ID NO: 124 - protein, 127 aa, synthetic construct
  REGION 1..127: note = An artificially synthesized peptide sequence
QVQLVESGGGLVQPGRSLRLSCAASGFTFSNAWMHWVRQAPGKGLEWVAQIKDRSSGYAAYYAPSVKGRFTISRDDSKNSIYLQMNSLKTEDTAVYYCRYVHYSRPFFGGKYGVDAWGQGTTVTVSS

SEQ ID NO: 125 - protein, 128 aa, synthetic construct
  REGION 1..128: note = An artificially synthesized peptide sequence
QVQLVESGGGLVQPGRSLRLSCAASGFTFSNAWMHWVRQAPGKGLEWVAQIKDKANQYNTYYAESVKGRFTISRDDSKNSIYLQMNSLKTEDTAVYYCRYVHYTTSFGFFYSFGVDAWGQGTTVTVSS

SEQ ID NO: 126 - protein, 128 aa, synthetic construct
  REGION 1..128: note = An artificially synthesized peptide sequence
QVQLVESGGGLVQPGRSLRLSCAASGFTFSNAWMHWVRQAPGKGLEWVAQIKDKSSGYATYYAESVKGRFTISRDDSKNSIYLQMNSLKTEDTAVYYCRYVHYTTFVGGYPSYGVDAWGQGTTVTVSS

SEQ ID NO: 127 - protein, 127 aa, synthetic construct
  REGION 1..127: note = An artificially synthesized peptide sequence
QVQLVESGGGLVQPGRSLRLSCAASGFTFSNAWMHWVRQAPGKGLEWVAQIKDRGNSYNAYYAESVKGRFTISRDDSKNSIYLQMNSLKTEDTAVYYCRYVHYTTTYSGYQYGVDAWGQGTTVTVSS

SEQ ID NO: 128 - protein, 127 aa, synthetic construct
  REGION 1..127: note = An artificially synthesized peptide sequence
QVQLVESGGGLVQPGRSLRLSCAASGFTFSNAWMHWVRQAPGKGLEWVAQIKDRQNNYATYYAESVKGRFTISRDDSKNSIYLQMNSLKTEDTAVYYCRYVHYTTYFGGSYGGVDAWGQGTTVTVSS

SEQ ID NO: 129 - protein, 128 aa, synthetic construct
  REGION 1..128: note = An artificially synthesized peptide sequence
QVQLVESGGGLVQPGRSLRLSCAASGFTFSNAWMHWVRQAPGKGLEWVAQIKDRQNQYATYYAESVKGRFTISRDDSKNSIYLQMNSLKTEDTAVYYCRYVHYTSFAGSGSSFGVDAWGQGTTVTVSS

SEQ ID NO: 130 - protein, 128 aa, synthetic construct
  REGION 1..128: note = An artificially synthesized peptide sequence
QVQLVESGGGLVQPGRSLRLSCAASGFTFSNAWMHWVRQAPGKGLEWVAQIKDRQQGYANYYAPSVKGRFTISRDDSKNSIYLQMNSLKTEDTAVYYCRYVHYTTSFDGSYQYGVDVWGQGTTVTVSS

SEQ ID NO: 131 - protein, 128 aa, synthetic construct
  REGION 1..128: note = An artificially synthesized peptide sequence
QVQLVESGGGLVQPGRSLRLSCAASGFTFSNAWMHWVRQAPGKGLEWVAQIKDKANGYNAYYAPSVKGRFTISRDDSKNSIYLQMNSLKTEDTAVYYCRYVHYTTFGFGLSYGGVDAWGQGTTVTVSS

SEQ ID NO: 132 - protein, 128 aa, synthetic construct
  REGION 1..128: note = An artificially synthesized peptide sequence
QVQLVESGGGLVQPGRSLRLSCAASGFTFSNAWMHWVRQAPGKGLEWVAQIKDRQNNYATYYAESVKGRFTISRDDSKNSIYLQMNSLKTEDTAVYYCRYVHYATYFSGLYKFGVDAWGQGTTVTVSS

SEQ ID NO: 133 - protein, 128 aa, synthetic construct
  REGION 1..128: note = An artificially synthesized peptide sequence
QVQLVESGGGLVQPGRSLRLSCAASGFTFSNAWMHWVRQAPGKGLEWVAQIKDRQNGYATYYAPSVKGRFTISRDDSKNSIYLQMNSLKTEDTAVYYCRYVHYTTYYGGYFQFGVDAWGQGTTVTVSS

SEQ ID NO: 134 - protein, 128 aa, synthetic construct
  REGION 1..128: note = An artificially synthesized peptide sequence
QVQLVESGGGLVQPGRSLRLSCAASGFTFSNAWMHWVRQAPGKGLEWVAQIKDKGNSYATYYAPSVKGRFTISRDDSKNSIYLQMNSLKTEDTAVYYCRYVHYTTVSFLGFKYGVDAWGQGTTVTVSS

SEQ ID NO: 135 - protein, 128 aa, synthetic construct
  REGION 1..128: note = An artificially synthesized peptide sequence
QVQLVESGGGLVQPGRSLRLSCAASGFTFSNAWMHWVRQAPGKGLEWVAQIKDRGNAYNAYYAESVKGRFTISRDDSKNSIYLQMNSLKTEDTAVYYCRYVHYASYAFGFFSYGVDAWGQGTTVTVSS

SEQ ID NO: 136 - protein, 471 aa, synthetic construct
  REGION 1..471: note = An artificially synthesized peptide sequence
QVQLVESGGGLVQPGRSLRLSCAASGFTFSNAWMHWVRQAPGKGLEWVAQIKDKGQQYAAYYAPSVKGRFTISRDGCRGDCLDSKNSIYLQMNSLKTEDTAVYYCRYVHYQTYSDGSFYFGVDAWGQGTTVTVSSASTKGPSVFPLAPSSKSTSGGTAALGCLVKDYFPEPVTVSWNSGALTSGVHTFPAVLQSSGLYSLSSVVTVPSSSLGTQTYICNVNHKPSNTKVDKKVEPKSCDKTHTCPPCPAPEAAGGPSVFLFPPKPKDTLMISRTPEVTCVVVDVSHEDPEVKFNWYVDGVEVHNAKTKPREEQYASTYRVVSVLTVLHQDWLNGKEYKCKVSNKALPAPIEKTISKAKGQPREPQVYTLPPSRCELTKNQVSLSCAVKGFYPSDIAVEWESNGQPENNYKTTPPVLDSDGSFFLVSKLTVDKSRWQQGNVFSCSVMHEALHNHYTQKSLSLSPDYKDDDDK